European Patent Application EP 4 745 239 A1, published May 20, 2026. Title: CFB抑制剂组合物及其应用. Applicant: 苏州炫景生物科技有限公司. The sequence listing filed with the application follows.

SEQUENCE LISTING (525 sequences)

SEQ ID NO: 1 - RNA, 19 nt, artificial sequence
  source 1..19: mol_type = genomic RNA
cctttatcttgggcctctt

SEQ ID NO: 2 - RNA, 19 nt, artificial sequence
  source 1..19: mol_type = genomic RNA
ggtgtgaccaccactccat

SEQ ID NO: 3 - RNA, 19 nt, artificial sequence
  source 1..19: mol_type = genomic RNA
gtagagatcaaaggcggct

SEQ ID NO: 4 - RNA, 19 nt, artificial sequence
  source 1..19: mol_type = genomic RNA
caaaggcggctccttccga

SEQ ID NO: 5 - RNA, 19 nt, artificial sequence
  source 1..19: mol_type = genomic RNA
aaggcggctccttccgact

SEQ ID NO: 6 - RNA, 19 nt, artificial sequence
  source 1..19: mol_type = genomic RNA
gcggctccttccgacttct

SEQ ID NO: 7 - RNA, 19 nt, artificial sequence
  source 1..19: mol_type = genomic RNA
gctccttccgacttctcca

SEQ ID NO: 8 - RNA, 19 nt, artificial sequence
  source 1..19: mol_type = genomic RNA
ctccttccgacttctccaa

SEQ ID NO: 9 - RNA, 19 nt, artificial sequence
  source 1..19: mol_type = genomic RNA
ccttccgacttctccaaga

SEQ ID NO: 10 - RNA, 19 nt, artificial sequence
  source 1..19: mol_type = genomic RNA
cttccgacttctccaagag

SEQ ID NO: 11 - RNA, 19 nt, artificial sequence
  source 1..19: mol_type = genomic RNA
gacttctccaagagggcca

SEQ ID NO: 12 - RNA, 19 nt, artificial sequence
  source 1..19: mol_type = genomic RNA
gccaggcactggagtacgt

SEQ ID NO: 13 - RNA, 19 nt, artificial sequence
  source 1..19: mol_type = genomic RNA
ggagtacgtgtgtccttct

SEQ ID NO: 14 - RNA, 19 nt, artificial sequence
  source 1..19: mol_type = genomic RNA
gtgtgtccttctggcttct

SEQ ID NO: 15 - RNA, 19 nt, artificial sequence
  source 1..19: mol_type = genomic RNA
ccttctggcttctacccgt

SEQ ID NO: 16 - RNA, 19 nt, artificial sequence
  source 1..19: mol_type = genomic RNA
cttctggcttctacccgta

SEQ ID NO: 17 - RNA, 19 nt, artificial sequence
  source 1..19: mol_type = genomic RNA
gcttctacccgtaccctgt

SEQ ID NO: 18 - RNA, 19 nt, artificial sequence
  source 1..19: mol_type = genomic RNA
cccgtaccctgtgcagaca

SEQ ID NO: 19 - RNA, 19 nt, artificial sequence
  source 1..19: mol_type = genomic RNA
cctgtgcagacacgtacct

SEQ ID NO: 20 - RNA, 19 nt, artificial sequence
  source 1..19: mol_type = genomic RNA
gcagacacgtacctgcaga

SEQ ID NO: 21 - RNA, 19 nt, artificial sequence
  source 1..19: mol_type = genomic RNA
cagacacgtacctgcagat

SEQ ID NO: 22 - RNA, 19 nt, artificial sequence
  source 1..19: mol_type = genomic RNA
acacgtacctgcagatcta

SEQ ID NO: 23 - RNA, 19 nt, artificial sequence
  source 1..19: mol_type = genomic RNA
cggggtcctggagcaccct

SEQ ID NO: 24 - RNA, 19 nt, artificial sequence
  source 1..19: mol_type = genomic RNA
ctggagcaccctgaagact

SEQ ID NO: 25 - RNA, 19 nt, artificial sequence
  source 1..19: mol_type = genomic RNA
ggagcaccctgaagactca

SEQ ID NO: 26 - RNA, 19 nt, artificial sequence
  source 1..19: mol_type = genomic RNA
gcaccctgaagactcaaga

SEQ ID NO: 27 - RNA, 19 nt, artificial sequence
  source 1..19: mol_type = genomic RNA
caggaaggcagagtgcaga

SEQ ID NO: 28 - RNA, 19 nt, artificial sequence
  source 1..19: mol_type = genomic RNA
aaggcagagtgcagagcaa

SEQ ID NO: 29 - RNA, 19 nt, artificial sequence
  source 1..19: mol_type = genomic RNA
gtgcagagcaatccactgt

SEQ ID NO: 30 - RNA, 19 nt, artificial sequence
  source 1..19: mol_type = genomic RNA
gaccacacgacttcgagaa

SEQ ID NO: 31 - RNA, 19 nt, artificial sequence
  source 1..19: mol_type = genomic RNA
ggtctccctactacaatgt

SEQ ID NO: 32 - RNA, 19 nt, artificial sequence
  source 1..19: mol_type = genomic RNA
cctactacaatgtgagtga

SEQ ID NO: 33 - RNA, 19 nt, artificial sequence
  source 1..19: mol_type = genomic RNA
ctactacaatgtgagtgat

SEQ ID NO: 34 - RNA, 19 nt, artificial sequence
  source 1..19: mol_type = genomic RNA
caatgtgagtgatgagatc

SEQ ID NO: 35 - RNA, 19 nt, artificial sequence
  source 1..19: mol_type = genomic RNA
gtgatgagatctctttcca

SEQ ID NO: 36 - RNA, 19 nt, artificial sequence
  source 1..19: mol_type = genomic RNA
gatgagatctctttccact

SEQ ID NO: 37 - RNA, 19 nt, artificial sequence
  source 1..19: mol_type = genomic RNA
gagatctctttccactgct

SEQ ID NO: 38 - RNA, 19 nt, artificial sequence
  source 1..19: mol_type = genomic RNA
agatctctttccactgcta

SEQ ID NO: 39 - RNA, 19 nt, artificial sequence
  source 1..19: mol_type = genomic RNA
gatctctttccactgctat

SEQ ID NO: 40 - RNA, 19 nt, artificial sequence
  source 1..19: mol_type = genomic RNA
gctatgacggttacactct

SEQ ID NO: 41 - RNA, 19 nt, artificial sequence
  source 1..19: mol_type = genomic RNA
ctgccaatcgcacctgcca

SEQ ID NO: 42 - RNA, 19 nt, artificial sequence
  source 1..19: mol_type = genomic RNA
aatcgcacctgccaagtga

SEQ ID NO: 43 - RNA, 19 nt, artificial sequence
  source 1..19: mol_type = genomic RNA
atcgcacctgccaagtgaa

SEQ ID NO: 44 - RNA, 19 nt, artificial sequence
  source 1..19: mol_type = genomic RNA
agtgaatggccgatggagt

SEQ ID NO: 45 - RNA, 19 nt, artificial sequence
  source 1..19: mol_type = genomic RNA
gaatggccgatggagtggg

SEQ ID NO: 46 - RNA, 19 nt, artificial sequence
  source 1..19: mol_type = genomic RNA
ccgatggagtgggcagaca

SEQ ID NO: 47 - RNA, 19 nt, artificial sequence
  source 1..19: mol_type = genomic RNA
atggagtgggcagacagcg

SEQ ID NO: 48 - RNA, 19 nt, artificial sequence
  source 1..19: mol_type = genomic RNA
ggagtgggcagacagcgat

SEQ ID NO: 49 - RNA, 19 nt, artificial sequence
  source 1..19: mol_type = genomic RNA
tgggcagacagcgatctgt

SEQ ID NO: 50 - RNA, 19 nt, artificial sequence
  source 1..19: mol_type = genomic RNA
ggcagacagcgatctgtga

SEQ ID NO: 51 - RNA, 19 nt, artificial sequence
  source 1..19: mol_type = genomic RNA
gcagacagcgatctgtgac

SEQ ID NO: 52 - RNA, 19 nt, artificial sequence
  source 1..19: mol_type = genomic RNA
cagacagcgatctgtgaca

SEQ ID NO: 53 - RNA, 19 nt, artificial sequence
  source 1..19: mol_type = genomic RNA
ggcacaaggaaggtgggca

SEQ ID NO: 54 - RNA, 19 nt, artificial sequence
  source 1..19: mol_type = genomic RNA
gcacaaggaaggtgggcag

SEQ ID NO: 55 - RNA, 19 nt, artificial sequence
  source 1..19: mol_type = genomic RNA
caaggaaggtgggcagcca

SEQ ID NO: 56 - RNA, 19 nt, artificial sequence
  source 1..19: mol_type = genomic RNA
gcagccagtaccgccttga

SEQ ID NO: 57 - RNA, 19 nt, artificial sequence
  source 1..19: mol_type = genomic RNA
cttgaagacagcgtcacct

SEQ ID NO: 58 - RNA, 19 nt, artificial sequence
  source 1..19: mol_type = genomic RNA
gacagcgtcacctaccact

SEQ ID NO: 59 - RNA, 19 nt, artificial sequence
  source 1..19: mol_type = genomic RNA
ccgggggcttaccctgcgt

SEQ ID NO: 60 - RNA, 19 nt, artificial sequence
  source 1..19: mol_type = genomic RNA
gcggcgaacgtgtcaggaa

SEQ ID NO: 61 - RNA, 19 nt, artificial sequence
  source 1..19: mol_type = genomic RNA
gcgaacgtgtcaggaaggt

SEQ ID NO: 62 - RNA, 19 nt, artificial sequence
  source 1..19: mol_type = genomic RNA
gtgtcaggaaggtggctct

SEQ ID NO: 63 - RNA, 19 nt, artificial sequence
  source 1..19: mol_type = genomic RNA
ggaaggtggctcttggagc

SEQ ID NO: 64 - RNA, 19 nt, artificial sequence
  source 1..19: mol_type = genomic RNA
aggtggctcttggagcggg

SEQ ID NO: 65 - RNA, 19 nt, artificial sequence
  source 1..19: mol_type = genomic RNA
gagcgggacggagccttcc

SEQ ID NO: 66 - RNA, 19 nt, artificial sequence
  source 1..19: mol_type = genomic RNA
gacggagccttcctgccaa

SEQ ID NO: 67 - RNA, 19 nt, artificial sequence
  source 1..19: mol_type = genomic RNA
gagccttcctgccaagact

SEQ ID NO: 68 - RNA, 19 nt, artificial sequence
  source 1..19: mol_type = genomic RNA
ccttcctgccaagactcct

SEQ ID NO: 69 - RNA, 19 nt, artificial sequence
  source 1..19: mol_type = genomic RNA
cttcctgccaagactcctt

SEQ ID NO: 70 - RNA, 19 nt, artificial sequence
  source 1..19: mol_type = genomic RNA
cctgccaagactccttcat

SEQ ID NO: 71 - RNA, 19 nt, artificial sequence
  source 1..19: mol_type = genomic RNA
gccaagactccttcatgta

SEQ ID NO: 72 - RNA, 19 nt, artificial sequence
  source 1..19: mol_type = genomic RNA
gactccttcatgtacgaca

SEQ ID NO: 73 - RNA, 19 nt, artificial sequence
  source 1..19: mol_type = genomic RNA
actccttcatgtacgacac

SEQ ID NO: 74 - RNA, 19 nt, artificial sequence
  source 1..19: mol_type = genomic RNA
ctccttcatgtacgacacc

SEQ ID NO: 75 - RNA, 19 nt, artificial sequence
  source 1..19: mol_type = genomic RNA
ggccgaagctttcctgtct

SEQ ID NO: 76 - RNA, 19 nt, artificial sequence
  source 1..19: mol_type = genomic RNA
gccgaagctttcctgtctt

SEQ ID NO: 77 - RNA, 19 nt, artificial sequence
  source 1..19: mol_type = genomic RNA
gctttcctgtcttccctga

SEQ ID NO: 78 - RNA, 19 nt, artificial sequence
  source 1..19: mol_type = genomic RNA
cctgacagagaccatagaa

SEQ ID NO: 79 - RNA, 19 nt, artificial sequence
  source 1..19: mol_type = genomic RNA
gacagagaccatagaagga

SEQ ID NO: 80 - RNA, 19 nt, artificial sequence
  source 1..19: mol_type = genomic RNA
cagagaccatagaaggagt

SEQ ID NO: 81 - RNA, 19 nt, artificial sequence
  source 1..19: mol_type = genomic RNA
gaccatagaaggagtcgat

SEQ ID NO: 82 - RNA, 19 nt, artificial sequence
  source 1..19: mol_type = genomic RNA
catagaaggagtcgatgct

SEQ ID NO: 83 - RNA, 19 nt, artificial sequence
  source 1..19: mol_type = genomic RNA
tagaaggagtcgatgctga

SEQ ID NO: 84 - RNA, 19 nt, artificial sequence
  source 1..19: mol_type = genomic RNA
aggagtcgatgctgaggat

SEQ ID NO: 85 - RNA, 19 nt, artificial sequence
  source 1..19: mol_type = genomic RNA
atgggcacggcccagggga

SEQ ID NO: 86 - RNA, 19 nt, artificial sequence
  source 1..19: mol_type = genomic RNA
gggaacaacagaagcggaa

SEQ ID NO: 87 - RNA, 19 nt, artificial sequence
  source 1..19: mol_type = genomic RNA
gaacaacagaagcggaaga

SEQ ID NO: 88 - RNA, 19 nt, artificial sequence
  source 1..19: mol_type = genomic RNA
caacagaagcggaagatcg

SEQ ID NO: 89 - RNA, 19 nt, artificial sequence
  source 1..19: mol_type = genomic RNA
ctggacccttcaggctcca

SEQ ID NO: 90 - RNA, 19 nt, artificial sequence
  source 1..19: mol_type = genomic RNA
ccttcaggctccatgaaca

SEQ ID NO: 91 - RNA, 19 nt, artificial sequence
  source 1..19: mol_type = genomic RNA
caggctccatgaacatcta

SEQ ID NO: 92 - RNA, 19 nt, artificial sequence
  source 1..19: mol_type = genomic RNA
gctccatgaacatctacct

SEQ ID NO: 93 - RNA, 19 nt, artificial sequence
  source 1..19: mol_type = genomic RNA
ccatgaacatctacctggt

SEQ ID NO: 94 - RNA, 19 nt, artificial sequence
  source 1..19: mol_type = genomic RNA
aacatctacctggtgctag

SEQ ID NO: 95 - RNA, 19 nt, artificial sequence
  source 1..19: mol_type = genomic RNA
tacctggtgctagatggat

SEQ ID NO: 96 - RNA, 19 nt, artificial sequence
  source 1..19: mol_type = genomic RNA
acctggtgctagatggatc

SEQ ID NO: 97 - RNA, 19 nt, artificial sequence
  source 1..19: mol_type = genomic RNA
cctggtgctagatggatca

SEQ ID NO: 98 - RNA, 19 nt, artificial sequence
  source 1..19: mol_type = genomic RNA
ctagatggatcagacagca

SEQ ID NO: 99 - RNA, 19 nt, artificial sequence
  source 1..19: mol_type = genomic RNA
tggatcagacagcattggg

SEQ ID NO: 100 - RNA, 19 nt, artificial sequence
  source 1..19: mol_type = genomic RNA
gccagcaacttcacaggag

SEQ ID NO: 101 - RNA, 19 nt, artificial sequence
  source 1..19: mol_type = genomic RNA
caacttcacaggagccaaa

SEQ ID NO: 102 - RNA, 19 nt, artificial sequence
  source 1..19: mol_type = genomic RNA
aaagtgtctagtcaactta

SEQ ID NO: 103 - RNA, 19 nt, artificial sequence
  source 1..19: mol_type = genomic RNA
aagtgtctagtcaacttaa

SEQ ID NO: 104 - RNA, 19 nt, artificial sequence
  source 1..19: mol_type = genomic RNA
agtgtctagtcaacttaat

SEQ ID NO: 105 - RNA, 19 nt, artificial sequence
  source 1..19: mol_type = genomic RNA
gtctagtcaacttaattga

SEQ ID NO: 106 - RNA, 19 nt, artificial sequence
  source 1..19: mol_type = genomic RNA
ctagtcaacttaattgaga

SEQ ID NO: 107 - RNA, 19 nt, artificial sequence
  source 1..19: mol_type = genomic RNA
ttgagaaggtggcaagtta

SEQ ID NO: 108 - RNA, 19 nt, artificial sequence
  source 1..19: mol_type = genomic RNA
gaaggtggcaagttatggt

SEQ ID NO: 109 - RNA, 19 nt, artificial sequence
  source 1..19: mol_type = genomic RNA
gtggcaagttatggtgtga

SEQ ID NO: 110 - RNA, 19 nt, artificial sequence
  source 1..19: mol_type = genomic RNA
agttatggtgtgaagccaa

SEQ ID NO: 111 - RNA, 19 nt, artificial sequence
  source 1..19: mol_type = genomic RNA
ggtgtgaagccaagatatg

SEQ ID NO: 112 - RNA, 19 nt, artificial sequence
  source 1..19: mol_type = genomic RNA
gaagccaagatatggtcta

SEQ ID NO: 113 - RNA, 19 nt, artificial sequence
  source 1..19: mol_type = genomic RNA
aagatatggtctagtgaca

SEQ ID NO: 114 - RNA, 19 nt, artificial sequence
  source 1..19: mol_type = genomic RNA
gatatggtctagtgacata

SEQ ID NO: 115 - RNA, 19 nt, artificial sequence
  source 1..19: mol_type = genomic RNA
ggtctagtgacatatgcca

SEQ ID NO: 116 - RNA, 19 nt, artificial sequence
  source 1..19: mol_type = genomic RNA
ctagtgacatatgccacat

SEQ ID NO: 117 - RNA, 19 nt, artificial sequence
  source 1..19: mol_type = genomic RNA
ccaaaatttgggtcaaagt

SEQ ID NO: 118 - RNA, 19 nt, artificial sequence
  source 1..19: mol_type = genomic RNA
gacagcagtaatgcagact

SEQ ID NO: 119 - RNA, 19 nt, artificial sequence
  source 1..19: mol_type = genomic RNA
gcagtaatgcagactgggt

SEQ ID NO: 120 - RNA, 19 nt, artificial sequence
  source 1..19: mol_type = genomic RNA
agtaatgcagactgggtca

SEQ ID NO: 121 - RNA, 19 nt, artificial sequence
  source 1..19: mol_type = genomic RNA
cagactgggtcacgaagca

SEQ ID NO: 122 - RNA, 19 nt, artificial sequence
  source 1..19: mol_type = genomic RNA
gggtcacgaagcagctcaa

SEQ ID NO: 123 - RNA, 19 nt, artificial sequence
  source 1..19: mol_type = genomic RNA
gcagctcaatgaaatcaat

SEQ ID NO: 124 - RNA, 19 nt, artificial sequence
  source 1..19: mol_type = genomic RNA
gctcaatgaaatcaattat

SEQ ID NO: 125 - RNA, 19 nt, artificial sequence
  source 1..19: mol_type = genomic RNA
caatgaaatcaattatgaa

SEQ ID NO: 126 - RNA, 19 nt, artificial sequence
  source 1..19: mol_type = genomic RNA
tcaattatgaagaccacaa

SEQ ID NO: 127 - RNA, 19 nt, artificial sequence
  source 1..19: mol_type = genomic RNA
atgaagaccacaagttgaa

SEQ ID NO: 128 - RNA, 19 nt, artificial sequence
  source 1..19: mol_type = genomic RNA
gaagaccacaagttgaagt

SEQ ID NO: 129 - RNA, 19 nt, artificial sequence
  source 1..19: mol_type = genomic RNA
cacaagttgaagtcaggga

SEQ ID NO: 130 - RNA, 19 nt, artificial sequence
  source 1..19: mol_type = genomic RNA
agttgaagtcagggactaa

SEQ ID NO: 131 - RNA, 19 nt, artificial sequence
  source 1..19: mol_type = genomic RNA
cagggactaacaccaagaa

SEQ ID NO: 132 - RNA, 19 nt, artificial sequence
  source 1..19: mol_type = genomic RNA
ctaacaccaagaaggccct

SEQ ID NO: 133 - RNA, 19 nt, artificial sequence
  source 1..19: mol_type = genomic RNA
caggcagtgtacagcatga

SEQ ID NO: 134 - RNA, 19 nt, artificial sequence
  source 1..19: mol_type = genomic RNA
gcagtgtacagcatgatga

SEQ ID NO: 135 - RNA, 19 nt, artificial sequence
  source 1..19: mol_type = genomic RNA
gtgtacagcatgatgagct

SEQ ID NO: 136 - RNA, 19 nt, artificial sequence
  source 1..19: mol_type = genomic RNA
cctgaaggctggaaccgca

SEQ ID NO: 137 - RNA, 19 nt, artificial sequence
  source 1..19: mol_type = genomic RNA
gcacccgccatgtcatcat

SEQ ID NO: 138 - RNA, 19 nt, artificial sequence
  source 1..19: mol_type = genomic RNA
cccgccatgtcatcatcct

SEQ ID NO: 139 - RNA, 19 nt, artificial sequence
  source 1..19: mol_type = genomic RNA
cgccatgtcatcatcctca

SEQ ID NO: 140 - RNA, 19 nt, artificial sequence
  source 1..19: mol_type = genomic RNA
gccatgtcatcatcctcat

SEQ ID NO: 141 - RNA, 19 nt, artificial sequence
  source 1..19: mol_type = genomic RNA
catgtcatcatcctcatga

SEQ ID NO: 142 - RNA, 19 nt, artificial sequence
  source 1..19: mol_type = genomic RNA
cctcatgactgatggattg

SEQ ID NO: 143 - RNA, 19 nt, artificial sequence
  source 1..19: mol_type = genomic RNA
tgactgatggattgcacaa

SEQ ID NO: 144 - RNA, 19 nt, artificial sequence
  source 1..19: mol_type = genomic RNA
ctgatggattgcacaacat

SEQ ID NO: 145 - RNA, 19 nt, artificial sequence
  source 1..19: mol_type = genomic RNA
cccaattactgtcattgat

SEQ ID NO: 146 - RNA, 19 nt, artificial sequence
  source 1..19: mol_type = genomic RNA
caattactgtcattgatga

SEQ ID NO: 147 - RNA, 19 nt, artificial sequence
  source 1..19: mol_type = genomic RNA
ccgggacttgctatacatt

SEQ ID NO: 148 - RNA, 19 nt, artificial sequence
  source 1..19: mol_type = genomic RNA
caagggaggattatctgga

SEQ ID NO: 149 - RNA, 19 nt, artificial sequence
  source 1..19: mol_type = genomic RNA
gggaggattatctggatgt

SEQ ID NO: 150 - RNA, 19 nt, artificial sequence
  source 1..19: mol_type = genomic RNA
aggattatctggatgtcta

SEQ ID NO: 151 - RNA, 19 nt, artificial sequence
  source 1..19: mol_type = genomic RNA
ggattatctggatgtctat

SEQ ID NO: 152 - RNA, 19 nt, artificial sequence
  source 1..19: mol_type = genomic RNA
tctggatgtctatgtgttt

SEQ ID NO: 153 - RNA, 19 nt, artificial sequence
  source 1..19: mol_type = genomic RNA
ctttggtgaaccaagtgaa

SEQ ID NO: 154 - RNA, 19 nt, artificial sequence
  source 1..19: mol_type = genomic RNA
tgaaccaagtgaacatcaa

SEQ ID NO: 155 - RNA, 19 nt, artificial sequence
  source 1..19: mol_type = genomic RNA
caagtgaacatcaatgctt

SEQ ID NO: 156 - RNA, 19 nt, artificial sequence
  source 1..19: mol_type = genomic RNA
aagtgaacatcaatgcttt

SEQ ID NO: 157 - RNA, 19 nt, artificial sequence
  source 1..19: mol_type = genomic RNA
gaacatcaatgctttggct

SEQ ID NO: 158 - RNA, 19 nt, artificial sequence
  source 1..19: mol_type = genomic RNA
cttccaagaaagacaatga

SEQ ID NO: 159 - RNA, 19 nt, artificial sequence
  source 1..19: mol_type = genomic RNA
ccaagaaagacaatgagca

SEQ ID NO: 160 - RNA, 19 nt, artificial sequence
  source 1..19: mol_type = genomic RNA
caagaaagacaatgagcaa

SEQ ID NO: 161 - RNA, 19 nt, artificial sequence
  source 1..19: mol_type = genomic RNA
agaaagacaatgagcaaca

SEQ ID NO: 162 - RNA, 19 nt, artificial sequence
  source 1..19: mol_type = genomic RNA
gaaagacaatgagcaacat

SEQ ID NO: 163 - RNA, 19 nt, artificial sequence
  source 1..19: mol_type = genomic RNA
caacatgtgttcaaagtca

SEQ ID NO: 164 - RNA, 19 nt, artificial sequence
  source 1..19: mol_type = genomic RNA
aacatgtgttcaaagtcaa

SEQ ID NO: 165 - RNA, 19 nt, artificial sequence
  source 1..19: mol_type = genomic RNA
gtgttcaaagtcaaggata

SEQ ID NO: 166 - RNA, 19 nt, artificial sequence
  source 1..19: mol_type = genomic RNA
tgttcaaagtcaaggatat

SEQ ID NO: 167 - RNA, 19 nt, artificial sequence
  source 1..19: mol_type = genomic RNA
caaagtcaaggatatggaa

SEQ ID NO: 168 - RNA, 19 nt, artificial sequence
  source 1..19: mol_type = genomic RNA
ggaaaacctggaagatgtt

SEQ ID NO: 169 - RNA, 19 nt, artificial sequence
  source 1..19: mol_type = genomic RNA
gatcgatgaaagccagtct

SEQ ID NO: 170 - RNA, 19 nt, artificial sequence
  source 1..19: mol_type = genomic RNA
gccagtctctgagtctctg

SEQ ID NO: 171 - RNA, 19 nt, artificial sequence
  source 1..19: mol_type = genomic RNA
ctctgagtctctgtggcat

SEQ ID NO: 172 - RNA, 19 nt, artificial sequence
  source 1..19: mol_type = genomic RNA
gagtctctgtggcatggtt

SEQ ID NO: 173 - RNA, 19 nt, artificial sequence
  source 1..19: mol_type = genomic RNA
gtggcatggtttgggaaca

SEQ ID NO: 174 - RNA, 19 nt, artificial sequence
  source 1..19: mol_type = genomic RNA
ggcatggtttgggaacaca

SEQ ID NO: 175 - RNA, 19 nt, artificial sequence
  source 1..19: mol_type = genomic RNA
gtaccgattaccacaagca

SEQ ID NO: 176 - RNA, 19 nt, artificial sequence
  source 1..19: mol_type = genomic RNA
gattaccacaagcaaccat

SEQ ID NO: 177 - RNA, 19 nt, artificial sequence
  source 1..19: mol_type = genomic RNA
ggcaggccaagatctcagt

SEQ ID NO: 178 - RNA, 19 nt, artificial sequence
  source 1..19: mol_type = genomic RNA
caggccaagatctcagtca

SEQ ID NO: 179 - RNA, 19 nt, artificial sequence
  source 1..19: mol_type = genomic RNA
ctcagtcattcgcccttca

SEQ ID NO: 180 - RNA, 19 nt, artificial sequence
  source 1..19: mol_type = genomic RNA
gctgtggtgtctgagtact

SEQ ID NO: 181 - RNA, 19 nt, artificial sequence
  source 1..19: mol_type = genomic RNA
gctgacagcagcacattgt

SEQ ID NO: 182 - RNA, 19 nt, artificial sequence
  source 1..19: mol_type = genomic RNA
cacattgtttcactgtgga

SEQ ID NO: 183 - RNA, 19 nt, artificial sequence
  source 1..19: mol_type = genomic RNA
gtttcactgtggatgacaa

SEQ ID NO: 184 - RNA, 19 nt, artificial sequence
  source 1..19: mol_type = genomic RNA
cactgtggatgacaaggaa

SEQ ID NO: 185 - RNA, 19 nt, artificial sequence
  source 1..19: mol_type = genomic RNA
ctgtggatgacaaggaaca

SEQ ID NO: 186 - RNA, 19 nt, artificial sequence
  source 1..19: mol_type = genomic RNA
gtggatgacaaggaacact

SEQ ID NO: 187 - RNA, 19 nt, artificial sequence
  source 1..19: mol_type = genomic RNA
acaaggaacactcaatcaa

SEQ ID NO: 188 - RNA, 19 nt, artificial sequence
  source 1..19: mol_type = genomic RNA
gaacactcaatcaaggtca

SEQ ID NO: 189 - RNA, 19 nt, artificial sequence
  source 1..19: mol_type = genomic RNA
gcgggacctggagatagaa

SEQ ID NO: 190 - RNA, 19 nt, artificial sequence
  source 1..19: mol_type = genomic RNA
gggacctggagatagaagt

SEQ ID NO: 191 - RNA, 19 nt, artificial sequence
  source 1..19: mol_type = genomic RNA
ggagatagaagtagtccta

SEQ ID NO: 192 - RNA, 19 nt, artificial sequence
  source 1..19: mol_type = genomic RNA
ctatttcaccccaactaca

SEQ ID NO: 193 - RNA, 19 nt, artificial sequence
  source 1..19: mol_type = genomic RNA
gaagcaggaattcctgaat

SEQ ID NO: 194 - RNA, 19 nt, artificial sequence
  source 1..19: mol_type = genomic RNA
caggaattcctgaatttta

SEQ ID NO: 195 - RNA, 19 nt, artificial sequence
  source 1..19: mol_type = genomic RNA
gaattcctgaattttatga

SEQ ID NO: 196 - RNA, 19 nt, artificial sequence
  source 1..19: mol_type = genomic RNA
ctgaattttatgactatga

SEQ ID NO: 197 - RNA, 19 nt, artificial sequence
  source 1..19: mol_type = genomic RNA
gttgccctgatcaagctca

SEQ ID NO: 198 - RNA, 19 nt, artificial sequence
  source 1..19: mol_type = genomic RNA
gccctgatcaagctcaaga

SEQ ID NO: 199 - RNA, 19 nt, artificial sequence
  source 1..19: mol_type = genomic RNA
ccctgatcaagctcaagaa

SEQ ID NO: 200 - RNA, 19 nt, artificial sequence
  source 1..19: mol_type = genomic RNA
cctgatcaagctcaagaat

SEQ ID NO: 201 - RNA, 19 nt, artificial sequence
  source 1..19: mol_type = genomic RNA
tgatcaagctcaagaataa

SEQ ID NO: 202 - RNA, 19 nt, artificial sequence
  source 1..19: mol_type = genomic RNA
gctcaagaataagctgaaa

SEQ ID NO: 203 - RNA, 19 nt, artificial sequence
  source 1..19: mol_type = genomic RNA
gccagactatcaggcccat

SEQ ID NO: 204 - RNA, 19 nt, artificial sequence
  source 1..19: mol_type = genomic RNA
ccagactatcaggcccatt

SEQ ID NO: 205 - RNA, 19 nt, artificial sequence
  source 1..19: mol_type = genomic RNA
cagactatcaggcccattt

SEQ ID NO: 206 - RNA, 19 nt, artificial sequence
  source 1..19: mol_type = genomic RNA
gactatcaggcccatttgt

SEQ ID NO: 207 - RNA, 19 nt, artificial sequence
  source 1..19: mol_type = genomic RNA
caccgagggaacaactcga

SEQ ID NO: 208 - RNA, 19 nt, artificial sequence
  source 1..19: mol_type = genomic RNA
cgagggaacaactcgagct

SEQ ID NO: 209 - RNA, 19 nt, artificial sequence
  source 1..19: mol_type = genomic RNA
gagggaacaactcgagctt

SEQ ID NO: 210 - RNA, 19 nt, artificial sequence
  source 1..19: mol_type = genomic RNA
gctttgaggcttcctccaa

SEQ ID NO: 211 - RNA, 19 nt, artificial sequence
  source 1..19: mol_type = genomic RNA
gcttcctccaactaccact

SEQ ID NO: 212 - RNA, 19 nt, artificial sequence
  source 1..19: mol_type = genomic RNA
cttcctccaactaccactt

SEQ ID NO: 213 - RNA, 19 nt, artificial sequence
  source 1..19: mol_type = genomic RNA
gctgctccctgcacaggat

SEQ ID NO: 214 - RNA, 19 nt, artificial sequence
  source 1..19: mol_type = genomic RNA
ccctgcacaggatatcaaa

SEQ ID NO: 215 - RNA, 19 nt, artificial sequence
  source 1..19: mol_type = genomic RNA
cacaggatatcaaagctct

SEQ ID NO: 216 - RNA, 19 nt, artificial sequence
  source 1..19: mol_type = genomic RNA
caggatatcaaagctctgt

SEQ ID NO: 217 - RNA, 19 nt, artificial sequence
  source 1..19: mol_type = genomic RNA
aggatatcaaagctctgtt

SEQ ID NO: 218 - RNA, 19 nt, artificial sequence
  source 1..19: mol_type = genomic RNA
ggatatcaaagctctgttt

SEQ ID NO: 219 - RNA, 19 nt, artificial sequence
  source 1..19: mol_type = genomic RNA
gatatcaaagctctgtttg

SEQ ID NO: 220 - RNA, 19 nt, artificial sequence
  source 1..19: mol_type = genomic RNA
ctctgtttgtgtctgagga

SEQ ID NO: 221 - RNA, 19 nt, artificial sequence
  source 1..19: mol_type = genomic RNA
ctgactcggaaggaggtct

SEQ ID NO: 222 - RNA, 19 nt, artificial sequence
  source 1..19: mol_type = genomic RNA
tgactcggaaggaggtcta

SEQ ID NO: 223 - RNA, 19 nt, artificial sequence
  source 1..19: mol_type = genomic RNA
gactcggaaggaggtctac

SEQ ID NO: 224 - RNA, 19 nt, artificial sequence
  source 1..19: mol_type = genomic RNA
ctcggaaggaggtctacat

SEQ ID NO: 225 - RNA, 19 nt, artificial sequence
  source 1..19: mol_type = genomic RNA
ggaaggaggtctacatcaa

SEQ ID NO: 226 - RNA, 19 nt, artificial sequence
  source 1..19: mol_type = genomic RNA
gaaggaggtctacatcaag

SEQ ID NO: 227 - RNA, 19 nt, artificial sequence
  source 1..19: mol_type = genomic RNA
ggaggtctacatcaagaat

SEQ ID NO: 228 - RNA, 19 nt, artificial sequence
  source 1..19: mol_type = genomic RNA
gaggtctacatcaagaatg

SEQ ID NO: 229 - RNA, 19 nt, artificial sequence
  source 1..19: mol_type = genomic RNA
caagaatggggataagaaa

SEQ ID NO: 230 - RNA, 19 nt, artificial sequence
  source 1..19: mol_type = genomic RNA
gctgtgagagagatgctca

SEQ ID NO: 231 - RNA, 19 nt, artificial sequence
  source 1..19: mol_type = genomic RNA
ctgtgagagagatgctcaa

SEQ ID NO: 232 - RNA, 19 nt, artificial sequence
  source 1..19: mol_type = genomic RNA
gtgagagagatgctcaata

SEQ ID NO: 233 - RNA, 19 nt, artificial sequence
  source 1..19: mol_type = genomic RNA
caggctatgacaaagtcaa

SEQ ID NO: 234 - RNA, 19 nt, artificial sequence
  source 1..19: mol_type = genomic RNA
gctatgacaaagtcaagga

SEQ ID NO: 235 - RNA, 19 nt, artificial sequence
  source 1..19: mol_type = genomic RNA
gacaaagtcaaggacatct

SEQ ID NO: 236 - RNA, 19 nt, artificial sequence
  source 1..19: mol_type = genomic RNA
gttcctttgtactggagga

SEQ ID NO: 237 - RNA, 19 nt, artificial sequence
  source 1..19: mol_type = genomic RNA
ctggaggagtgagtcccta

SEQ ID NO: 238 - RNA, 19 nt, artificial sequence
  source 1..19: mol_type = genomic RNA
cttgatagttcacaagaga

SEQ ID NO: 239 - RNA, 19 nt, artificial sequence
  source 1..19: mol_type = genomic RNA
gttcacaagagaagtcgtt

SEQ ID NO: 240 - RNA, 19 nt, artificial sequence
  source 1..19: mol_type = genomic RNA
cacaagagaagtcgtttca

SEQ ID NO: 241 - RNA, 19 nt, artificial sequence
  source 1..19: mol_type = genomic RNA
caagagaagtcgtttcatt

SEQ ID NO: 242 - RNA, 19 nt, artificial sequence
  source 1..19: mol_type = genomic RNA
agagaagtcgtttcattca

SEQ ID NO: 243 - RNA, 19 nt, artificial sequence
  source 1..19: mol_type = genomic RNA
gagaagtcgtttcattcaa

SEQ ID NO: 244 - RNA, 19 nt, artificial sequence
  source 1..19: mol_type = genomic RNA
gaagtcgtttcattcaagt

SEQ ID NO: 245 - RNA, 19 nt, artificial sequence
  source 1..19: mol_type = genomic RNA
gtttcattcaagttggtgt

SEQ ID NO: 246 - RNA, 19 nt, artificial sequence
  source 1..19: mol_type = genomic RNA
cccgagactttcacatcaa

SEQ ID NO: 247 - RNA, 19 nt, artificial sequence
  source 1..19: mol_type = genomic RNA
gagactttcacatcaacct

SEQ ID NO: 248 - RNA, 19 nt, artificial sequence
  source 1..19: mol_type = genomic RNA
gactttcacatcaacctct

SEQ ID NO: 249 - RNA, 19 nt, artificial sequence
  source 1..19: mol_type = genomic RNA
cctggctgaaggagaaact

SEQ ID NO: 250 - RNA, 19 nt, artificial sequence
  source 1..19: mol_type = genomic RNA
ggctgaaggagaaactcca

SEQ ID NO: 251 - RNA, 19 nt, artificial sequence
  source 1..19: mol_type = genomic RNA
gctgaaggagaaactccaa

SEQ ID NO: 252 - RNA, 19 nt, artificial sequence
  source 1..19: mol_type = genomic RNA
gaaggagaaactccaagat

SEQ ID NO: 253 - RNA, 19 nt, artificial sequence
  source 1..19: mol_type = genomic RNA
gaaactccaagatgaggat

SEQ ID NO: 254 - RNA, 19 nt, artificial sequence
  source 1..19: mol_type = genomic RNA
gaggatttgggttttctat

SEQ ID NO: 255 - RNA, 19 nt, artificial sequence
  source 1..19: mol_type = genomic RNA
ggatttgggttttctataa

SEQ ID NO: 256 - RNA, 21 nt, artificial sequence
  source 1..21: mol_type = genomic RNA
aagaggcccaagataaagggc

SEQ ID NO: 257 - RNA, 21 nt, artificial sequence
  source 1..21: mol_type = genomic RNA
atggagtggtggtcacacctc

SEQ ID NO: 258 - RNA, 21 nt, artificial sequence
  source 1..21: mol_type = genomic RNA
agccgcctttgatctctaccc

SEQ ID NO: 259 - RNA, 21 nt, artificial sequence
  source 1..21: mol_type = genomic RNA
tcggaaggagccgcctttgat

SEQ ID NO: 260 - RNA, 21 nt, artificial sequence
  source 1..21: mol_type = genomic RNA
agtcggaaggagccgcctttg

SEQ ID NO: 261 - RNA, 21 nt, artificial sequence
  source 1..21: mol_type = genomic RNA
agaagtcggaaggagccgcct

SEQ ID NO: 262 - RNA, 21 nt, artificial sequence
  source 1..21: mol_type = genomic RNA
tggagaagtcggaaggagccg

SEQ ID NO: 263 - RNA, 21 nt, artificial sequence
  source 1..21: mol_type = genomic RNA
ttggagaagtcggaaggagcc

SEQ ID NO: 264 - RNA, 21 nt, artificial sequence
  source 1..21: mol_type = genomic RNA
tcttggagaagtcggaaggag

SEQ ID NO: 265 - RNA, 21 nt, artificial sequence
  source 1..21: mol_type = genomic RNA
ctcttggagaagtcggaagga

SEQ ID NO: 266 - RNA, 21 nt, artificial sequence
  source 1..21: mol_type = genomic RNA
tggccctcttggagaagtcgg

SEQ ID NO: 267 - RNA, 21 nt, artificial sequence
  source 1..21: mol_type = genomic RNA
acgtactccagtgcctggccc

SEQ ID NO: 268 - RNA, 21 nt, artificial sequence
  source 1..21: mol_type = genomic RNA
agaaggacacacgtactccag

SEQ ID NO: 269 - RNA, 21 nt, artificial sequence
  source 1..21: mol_type = genomic RNA
agaagccagaaggacacacgt

SEQ ID NO: 270 - RNA, 21 nt, artificial sequence
  source 1..21: mol_type = genomic RNA
acgggtagaagccagaaggac

SEQ ID NO: 271 - RNA, 21 nt, artificial sequence
  source 1..21: mol_type = genomic RNA
tacgggtagaagccagaagga

SEQ ID NO: 272 - RNA, 21 nt, artificial sequence
  source 1..21: mol_type = genomic RNA
acagggtacgggtagaagcca

SEQ ID NO: 273 - RNA, 21 nt, artificial sequence
  source 1..21: mol_type = genomic RNA
tgtctgcacagggtacgggta

SEQ ID NO: 274 - RNA, 21 nt, artificial sequence
  source 1..21: mol_type = genomic RNA
aggtacgtgtctgcacagggt

SEQ ID NO: 275 - RNA, 21 nt, artificial sequence
  source 1..21: mol_type = genomic RNA
tctgcaggtacgtgtctgcac

SEQ ID NO: 276 - RNA, 21 nt, artificial sequence
  source 1..21: mol_type = genomic RNA
atctgcaggtacgtgtctgca

SEQ ID NO: 277 - RNA, 21 nt, artificial sequence
  source 1..21: mol_type = genomic RNA
tagatctgcaggtacgtgtct

SEQ ID NO: 278 - RNA, 21 nt, artificial sequence
  source 1..21: mol_type = genomic RNA
agggtgctccaggaccccgta

SEQ ID NO: 279 - RNA, 21 nt, artificial sequence
  source 1..21: mol_type = genomic RNA
agtcttcagggtgctccagga

SEQ ID NO: 280 - RNA, 21 nt, artificial sequence
  source 1..21: mol_type = genomic RNA
tgagtcttcagggtgctccag

SEQ ID NO: 281 - RNA, 21 nt, artificial sequence
  source 1..21: mol_type = genomic RNA
tcttgagtcttcagggtgctc

SEQ ID NO: 282 - RNA, 21 nt, artificial sequence
  source 1..21: mol_type = genomic RNA
tctgcactctgccttcctgac

SEQ ID NO: 283 - RNA, 21 nt, artificial sequence
  source 1..21: mol_type = genomic RNA
ttgctctgcactctgccttcc

SEQ ID NO: 284 - RNA, 21 nt, artificial sequence
  source 1..21: mol_type = genomic RNA
acagtggattgctctgcactc

SEQ ID NO: 285 - RNA, 21 nt, artificial sequence
  source 1..21: mol_type = genomic RNA
ttctcgaagtcgtgtggtctt

SEQ ID NO: 286 - RNA, 21 nt, artificial sequence
  source 1..21: mol_type = genomic RNA
acattgtagtagggagaccgg

SEQ ID NO: 287 - RNA, 21 nt, artificial sequence
  source 1..21: mol_type = genomic RNA
tcactcacattgtagtaggga

SEQ ID NO: 288 - RNA, 21 nt, artificial sequence
  source 1..21: mol_type = genomic RNA
atcactcacattgtagtaggg

SEQ ID NO: 289 - RNA, 21 nt, artificial sequence
  source 1..21: mol_type = genomic RNA
gatctcatcactcacattgta

SEQ ID NO: 290 - RNA, 21 nt, artificial sequence
  source 1..21: mol_type = genomic RNA
tggaaagagatctcatcactc

SEQ ID NO: 291 - RNA, 21 nt, artificial sequence
  source 1..21: mol_type = genomic RNA
agtggaaagagatctcatcac

SEQ ID NO: 292 - RNA, 21 nt, artificial sequence
  source 1..21: mol_type = genomic RNA
agcagtggaaagagatctcat

SEQ ID NO: 293 - RNA, 21 nt, artificial sequence
  source 1..21: mol_type = genomic RNA
tagcagtggaaagagatctca

SEQ ID NO: 294 - RNA, 21 nt, artificial sequence
  source 1..21: mol_type = genomic RNA
atagcagtggaaagagatctc

SEQ ID NO: 295 - RNA, 21 nt, artificial sequence
  source 1..21: mol_type = genomic RNA
agagtgtaaccgtcatagcag

SEQ ID NO: 296 - RNA, 21 nt, artificial sequence
  source 1..21: mol_type = genomic RNA
tggcaggtgcgattggcagag

SEQ ID NO: 297 - RNA, 21 nt, artificial sequence
  source 1..21: mol_type = genomic RNA
tcacttggcaggtgcgattgg

SEQ ID NO: 298 - RNA, 21 nt, artificial sequence
  source 1..21: mol_type = genomic RNA
ttcacttggcaggtgcgattg

SEQ ID NO: 299 - RNA, 21 nt, artificial sequence
  source 1..21: mol_type = genomic RNA
actccatcggccattcacttg

SEQ ID NO: 300 - RNA, 21 nt, artificial sequence
  source 1..21: mol_type = genomic RNA
cccactccatcggccattcac

SEQ ID NO: 301 - RNA, 21 nt, artificial sequence
  source 1..21: mol_type = genomic RNA
tgtctgcccactccatcggcc

SEQ ID NO: 302 - RNA, 21 nt, artificial sequence
  source 1..21: mol_type = genomic RNA
cgctgtctgcccactccatcg

SEQ ID NO: 303 - RNA, 21 nt, artificial sequence
  source 1..21: mol_type = genomic RNA
atcgctgtctgcccactccat

SEQ ID NO: 304 - RNA, 21 nt, artificial sequence
  source 1..21: mol_type = genomic RNA
acagatcgctgtctgcccact

SEQ ID NO: 305 - RNA, 21 nt, artificial sequence
  source 1..21: mol_type = genomic RNA
tcacagatcgctgtctgccca

SEQ ID NO: 306 - RNA, 21 nt, artificial sequence
  source 1..21: mol_type = genomic RNA
gtcacagatcgctgtctgccc

SEQ ID NO: 307 - RNA, 21 nt, artificial sequence
  source 1..21: mol_type = genomic RNA
tgtcacagatcgctgtctgcc

SEQ ID NO: 308 - RNA, 21 nt, artificial sequence
  source 1..21: mol_type = genomic RNA
tgcccaccttccttgtgccaa

SEQ ID NO: 309 - RNA, 21 nt, artificial sequence
  source 1..21: mol_type = genomic RNA
ctgcccaccttccttgtgcca

SEQ ID NO: 310 - RNA, 21 nt, artificial sequence
  source 1..21: mol_type = genomic RNA
tggctgcccaccttccttgtg

SEQ ID NO: 311 - RNA, 21 nt, artificial sequence
  source 1..21: mol_type = genomic RNA
tcaaggcggtactggctgccc

SEQ ID NO: 312 - RNA, 21 nt, artificial sequence
  source 1..21: mol_type = genomic RNA
aggtgacgctgtcttcaaggc

SEQ ID NO: 313 - RNA, 21 nt, artificial sequence
  source 1..21: mol_type = genomic RNA
agtggtaggtgacgctgtctt

SEQ ID NO: 314 - RNA, 21 nt, artificial sequence
  source 1..21: mol_type = genomic RNA
acgcagggtaagcccccggct

SEQ ID NO: 315 - RNA, 21 nt, artificial sequence
  source 1..21: mol_type = genomic RNA
ttcctgacacgttcgccgctg

SEQ ID NO: 316 - RNA, 21 nt, artificial sequence
  source 1..21: mol_type = genomic RNA
accttcctgacacgttcgccg

SEQ ID NO: 317 - RNA, 21 nt, artificial sequence
  source 1..21: mol_type = genomic RNA
agagccaccttcctgacacgt

SEQ ID NO: 318 - RNA, 21 nt, artificial sequence
  source 1..21: mol_type = genomic RNA
gctccaagagccaccttcctg

SEQ ID NO: 319 - RNA, 21 nt, artificial sequence
  source 1..21: mol_type = genomic RNA
cccgctccaagagccaccttc

SEQ ID NO: 320 - RNA, 21 nt, artificial sequence
  source 1..21: mol_type = genomic RNA
ggaaggctccgtcccgctcca

SEQ ID NO: 321 - RNA, 21 nt, artificial sequence
  source 1..21: mol_type = genomic RNA
ttggcaggaaggctccgtccc

SEQ ID NO: 322 - RNA, 21 nt, artificial sequence
  source 1..21: mol_type = genomic RNA
agtcttggcaggaaggctccg

SEQ ID NO: 323 - RNA, 21 nt, artificial sequence
  source 1..21: mol_type = genomic RNA
aggagtcttggcaggaaggct

SEQ ID NO: 324 - RNA, 21 nt, artificial sequence
  source 1..21: mol_type = genomic RNA
aaggagtcttggcaggaaggc

SEQ ID NO: 325 - RNA, 21 nt, artificial sequence
  source 1..21: mol_type = genomic RNA
atgaaggagtcttggcaggaa

SEQ ID NO: 326 - RNA, 21 nt, artificial sequence
  source 1..21: mol_type = genomic RNA
tacatgaaggagtcttggcag

SEQ ID NO: 327 - RNA, 21 nt, artificial sequence
  source 1..21: mol_type = genomic RNA
tgtcgtacatgaaggagtctt

SEQ ID NO: 328 - RNA, 21 nt, artificial sequence
  source 1..21: mol_type = genomic RNA
gtgtcgtacatgaaggagtct

SEQ ID NO: 329 - RNA, 21 nt, artificial sequence
  source 1..21: mol_type = genomic RNA
ggtgtcgtacatgaaggagtc

SEQ ID NO: 330 - RNA, 21 nt, artificial sequence
  source 1..21: mol_type = genomic RNA
agacaggaaagcttcggccac

SEQ ID NO: 331 - RNA, 21 nt, artificial sequence
  source 1..21: mol_type = genomic RNA
aagacaggaaagcttcggcca

SEQ ID NO: 332 - RNA, 21 nt, artificial sequence
  source 1..21: mol_type = genomic RNA
tcagggaagacaggaaagctt

SEQ ID NO: 333 - RNA, 21 nt, artificial sequence
  source 1..21: mol_type = genomic RNA
ttctatggtctctgtcaggga

SEQ ID NO: 334 - RNA, 21 nt, artificial sequence
  source 1..21: mol_type = genomic RNA
tccttctatggtctctgtcag

SEQ ID NO: 335 - RNA, 21 nt, artificial sequence
  source 1..21: mol_type = genomic RNA
actccttctatggtctctgtc

SEQ ID NO: 336 - RNA, 21 nt, artificial sequence
  source 1..21: mol_type = genomic RNA
atcgactccttctatggtctc

SEQ ID NO: 337 - RNA, 21 nt, artificial sequence
  source 1..21: mol_type = genomic RNA
agcatcgactccttctatggt

SEQ ID NO: 338 - RNA, 21 nt, artificial sequence
  source 1..21: mol_type = genomic RNA
tcagcatcgactccttctatg

SEQ ID NO: 339 - RNA, 21 nt, artificial sequence
  source 1..21: mol_type = genomic RNA
atcctcagcatcgactccttc

SEQ ID NO: 340 - RNA, 21 nt, artificial sequence
  source 1..21: mol_type = genomic RNA
tcccctgggccgtgcccatcc

SEQ ID NO: 341 - RNA, 21 nt, artificial sequence
  source 1..21: mol_type = genomic RNA
ttccgcttctgttgttcccct

SEQ ID NO: 342 - RNA, 21 nt, artificial sequence
  source 1..21: mol_type = genomic RNA
tcttccgcttctgttgttccc

SEQ ID NO: 343 - RNA, 21 nt, artificial sequence
  source 1..21: mol_type = genomic RNA
cgatcttccgcttctgttgtt

SEQ ID NO: 344 - RNA, 21 nt, artificial sequence
  source 1..21: mol_type = genomic RNA
tggagcctgaagggtccagga

SEQ ID NO: 345 - RNA, 21 nt, artificial sequence
  source 1..21: mol_type = genomic RNA
tgttcatggagcctgaagggt

SEQ ID NO: 346 - RNA, 21 nt, artificial sequence
  source 1..21: mol_type = genomic RNA
tagatgttcatggagcctgaa

SEQ ID NO: 347 - RNA, 21 nt, artificial sequence
  source 1..21: mol_type = genomic RNA
aggtagatgttcatggagcct

SEQ ID NO: 348 - RNA, 21 nt, artificial sequence
  source 1..21: mol_type = genomic RNA
accaggtagatgttcatggag

SEQ ID NO: 349 - RNA, 21 nt, artificial sequence
  source 1..21: mol_type = genomic RNA
ctagcaccaggtagatgttca

SEQ ID NO: 350 - RNA, 21 nt, artificial sequence
  source 1..21: mol_type = genomic RNA
atccatctagcaccaggtaga

SEQ ID NO: 351 - RNA, 21 nt, artificial sequence
  source 1..21: mol_type = genomic RNA
gatccatctagcaccaggtag

SEQ ID NO: 352 - RNA, 21 nt, artificial sequence
  source 1..21: mol_type = genomic RNA
tgatccatctagcaccaggta

SEQ ID NO: 353 - RNA, 21 nt, artificial sequence
  source 1..21: mol_type = genomic RNA
tgctgtctgatccatctagca

SEQ ID NO: 354 - RNA, 21 nt, artificial sequence
  source 1..21: mol_type = genomic RNA
cccaatgctgtctgatccatc

SEQ ID NO: 355 - RNA, 21 nt, artificial sequence
  source 1..21: mol_type = genomic RNA
ctcctgtgaagttgctggccc

SEQ ID NO: 356 - RNA, 21 nt, artificial sequence
  source 1..21: mol_type = genomic RNA
tttggctcctgtgaagttgct

SEQ ID NO: 357 - RNA, 21 nt, artificial sequence
  source 1..21: mol_type = genomic RNA
taagttgactagacacttttt

SEQ ID NO: 358 - RNA, 21 nt, artificial sequence
  source 1..21: mol_type = genomic RNA
ttaagttgactagacactttt

SEQ ID NO: 359 - RNA, 21 nt, artificial sequence
  source 1..21: mol_type = genomic RNA
attaagttgactagacacttt

SEQ ID NO: 360 - RNA, 21 nt, artificial sequence
  source 1..21: mol_type = genomic RNA
tcaattaagttgactagacac

SEQ ID NO: 361 - RNA, 21 nt, artificial sequence
  source 1..21: mol_type = genomic RNA
tctcaattaagttgactagac

SEQ ID NO: 362 - RNA, 21 nt, artificial sequence
  source 1..21: mol_type = genomic RNA
taacttgccaccttctcaatt

SEQ ID NO: 363 - RNA, 21 nt, artificial sequence
  source 1..21: mol_type = genomic RNA
accataacttgccaccttctc

SEQ ID NO: 364 - RNA, 21 nt, artificial sequence
  source 1..21: mol_type = genomic RNA
tcacaccataacttgccacct

SEQ ID NO: 365 - RNA, 21 nt, artificial sequence
  source 1..21: mol_type = genomic RNA
ttggcttcacaccataacttg

SEQ ID NO: 366 - RNA, 21 nt, artificial sequence
  source 1..21: mol_type = genomic RNA
catatcttggcttcacaccat

SEQ ID NO: 367 - RNA, 21 nt, artificial sequence
  source 1..21: mol_type = genomic RNA
tagaccatatcttggcttcac

SEQ ID NO: 368 - RNA, 21 nt, artificial sequence
  source 1..21: mol_type = genomic RNA
tgtcactagaccatatcttgg

SEQ ID NO: 369 - RNA, 21 nt, artificial sequence
  source 1..21: mol_type = genomic RNA
tatgtcactagaccatatctt

SEQ ID NO: 370 - RNA, 21 nt, artificial sequence
  source 1..21: mol_type = genomic RNA
tggcatatgtcactagaccat

SEQ ID NO: 371 - RNA, 21 nt, artificial sequence
  source 1..21: mol_type = genomic RNA
atgtggcatatgtcactagac

SEQ ID NO: 372 - RNA, 21 nt, artificial sequence
  source 1..21: mol_type = genomic RNA
actttgacccaaattttgggg

SEQ ID NO: 373 - RNA, 21 nt, artificial sequence
  source 1..21: mol_type = genomic RNA
agtctgcattactgctgtctg

SEQ ID NO: 374 - RNA, 21 nt, artificial sequence
  source 1..21: mol_type = genomic RNA
acccagtctgcattactgctg

SEQ ID NO: 375 - RNA, 21 nt, artificial sequence
  source 1..21: mol_type = genomic RNA
tgacccagtctgcattactgc

SEQ ID NO: 376 - RNA, 21 nt, artificial sequence
  source 1..21: mol_type = genomic RNA
tgcttcgtgacccagtctgca

SEQ ID NO: 377 - RNA, 21 nt, artificial sequence
  source 1..21: mol_type = genomic RNA
ttgagctgcttcgtgacccag

SEQ ID NO: 378 - RNA, 21 nt, artificial sequence
  source 1..21: mol_type = genomic RNA
attgatttcattgagctgctt

SEQ ID NO: 379 - RNA, 21 nt, artificial sequence
  source 1..21: mol_type = genomic RNA
ataattgatttcattgagctg

SEQ ID NO: 380 - RNA, 21 nt, artificial sequence
  source 1..21: mol_type = genomic RNA
ttcataattgatttcattgag

SEQ ID NO: 381 - RNA, 21 nt, artificial sequence
  source 1..21: mol_type = genomic RNA
ttgtggtcttcataattgatt

SEQ ID NO: 382 - RNA, 21 nt, artificial sequence
  source 1..21: mol_type = genomic RNA
ttcaacttgtggtcttcataa

SEQ ID NO: 383 - RNA, 21 nt, artificial sequence
  source 1..21: mol_type = genomic RNA
acttcaacttgtggtcttcat

SEQ ID NO: 384 - RNA, 21 nt, artificial sequence
  source 1..21: mol_type = genomic RNA
tccctgacttcaacttgtggt

SEQ ID NO: 385 - RNA, 21 nt, artificial sequence
  source 1..21: mol_type = genomic RNA
ttagtccctgacttcaacttg

SEQ ID NO: 386 - RNA, 21 nt, artificial sequence
  source 1..21: mol_type = genomic RNA
ttcttggtgttagtccctgac

SEQ ID NO: 387 - RNA, 21 nt, artificial sequence
  source 1..21: mol_type = genomic RNA
agggccttcttggtgttagtc

SEQ ID NO: 388 - RNA, 21 nt, artificial sequence
  source 1..21: mol_type = genomic RNA
tcatgctgtacactgcctgga

SEQ ID NO: 389 - RNA, 21 nt, artificial sequence
  source 1..21: mol_type = genomic RNA
tcatcatgctgtacactgcct

SEQ ID NO: 390 - RNA, 21 nt, artificial sequence
  source 1..21: mol_type = genomic RNA
agctcatcatgctgtacactg

SEQ ID NO: 391 - RNA, 21 nt, artificial sequence
  source 1..21: mol_type = genomic RNA
tgcggttccagccttcaggag

SEQ ID NO: 392 - RNA, 21 nt, artificial sequence
  source 1..21: mol_type = genomic RNA
atgatgacatggcgggtgcgg

SEQ ID NO: 393 - RNA, 21 nt, artificial sequence
  source 1..21: mol_type = genomic RNA
aggatgatgacatggcgggtg

SEQ ID NO: 394 - RNA, 21 nt, artificial sequence
  source 1..21: mol_type = genomic RNA
tgaggatgatgacatggcggg

SEQ ID NO: 395 - RNA, 21 nt, artificial sequence
  source 1..21: mol_type = genomic RNA
atgaggatgatgacatggcgg

SEQ ID NO: 396 - RNA, 21 nt, artificial sequence
  source 1..21: mol_type = genomic RNA
tcatgaggatgatgacatggc

SEQ ID NO: 397 - RNA, 21 nt, artificial sequence
  source 1..21: mol_type = genomic RNA
caatccatcagtcatgaggat

SEQ ID NO: 398 - RNA, 21 nt, artificial sequence
  source 1..21: mol_type = genomic RNA
ttgtgcaatccatcagtcatg

SEQ ID NO: 399 - RNA, 21 nt, artificial sequence
  source 1..21: mol_type = genomic RNA
atgttgtgcaatccatcagtc

SEQ ID NO: 400 - RNA, 21 nt, artificial sequence
  source 1..21: mol_type = genomic RNA
atcaatgacagtaattgggtc

SEQ ID NO: 401 - RNA, 21 nt, artificial sequence
  source 1..21: mol_type = genomic RNA
tcatcaatgacagtaattggg

SEQ ID NO: 402 - RNA, 21 nt, artificial sequence
  source 1..21: mol_type = genomic RNA
aatgtatagcaagtcccggat

SEQ ID NO: 403 - RNA, 21 nt, artificial sequence
  source 1..21: mol_type = genomic RNA
tccagataatcctcccttggg

SEQ ID NO: 404 - RNA, 21 nt, artificial sequence
  source 1..21: mol_type = genomic RNA
acatccagataatcctccctt

SEQ ID NO: 405 - RNA, 21 nt, artificial sequence
  source 1..21: mol_type = genomic RNA
tagacatccagataatcctcc

SEQ ID NO: 406 - RNA, 21 nt, artificial sequence
  source 1..21: mol_type = genomic RNA
atagacatccagataatcctc

SEQ ID NO: 407 - RNA, 21 nt, artificial sequence
  source 1..21: mol_type = genomic RNA
aaacacatagacatccagata

SEQ ID NO: 408 - RNA, 21 nt, artificial sequence
  source 1..21: mol_type = genomic RNA
ttcacttggttcaccaaaggc

SEQ ID NO: 409 - RNA, 21 nt, artificial sequence
  source 1..21: mol_type = genomic RNA
ttgatgttcacttggttcacc

SEQ ID NO: 410 - RNA, 21 nt, artificial sequence
  source 1..21: mol_type = genomic RNA
aagcattgatgttcacttggt

SEQ ID NO: 411 - RNA, 21 nt, artificial sequence
  source 1..21: mol_type = genomic RNA
aaagcattgatgttcacttgg

SEQ ID NO: 412 - RNA, 21 nt, artificial sequence
  source 1..21: mol_type = genomic RNA
agccaaagcattgatgttcac

SEQ ID NO: 413 - RNA, 21 nt, artificial sequence
  source 1..21: mol_type = genomic RNA
tcattgtctttcttggaagcc

SEQ ID NO: 414 - RNA, 21 nt, artificial sequence
  source 1..21: mol_type = genomic RNA
tgctcattgtctttcttggaa

SEQ ID NO: 415 - RNA, 21 nt, artificial sequence
  source 1..21: mol_type = genomic RNA
ttgctcattgtctttcttgga

SEQ ID NO: 416 - RNA, 21 nt, artificial sequence
  source 1..21: mol_type = genomic RNA
tgttgctcattgtctttcttg

SEQ ID NO: 417 - RNA, 21 nt, artificial sequence
  source 1..21: mol_type = genomic RNA
atgttgctcattgtctttctt

SEQ ID NO: 418 - RNA, 21 nt, artificial sequence
  source 1..21: mol_type = genomic RNA
tgactttgaacacatgttgct

SEQ ID NO: 419 - RNA, 21 nt, artificial sequence
  source 1..21: mol_type = genomic RNA
ttgactttgaacacatgttgc

SEQ ID NO: 420 - RNA, 21 nt, artificial sequence
  source 1..21: mol_type = genomic RNA
tatccttgactttgaacacat

SEQ ID NO: 421 - RNA, 21 nt, artificial sequence
  source 1..21: mol_type = genomic RNA
atatccttgactttgaacaca

SEQ ID NO: 422 - RNA, 21 nt, artificial sequence
  source 1..21: mol_type = genomic RNA
ttccatatccttgactttgaa

SEQ ID NO: 423 - RNA, 21 nt, artificial sequence
  source 1..21: mol_type = genomic RNA
aacatcttccaggttttccat

SEQ ID NO: 424 - RNA, 21 nt, artificial sequence
  source 1..21: mol_type = genomic RNA
agactggctttcatcgatcat

SEQ ID NO: 425 - RNA, 21 nt, artificial sequence
  source 1..21: mol_type = genomic RNA
cagagactcagagactggctt

SEQ ID NO: 426 - RNA, 21 nt, artificial sequence
  source 1..21: mol_type = genomic RNA
atgccacagagactcagagac

SEQ ID NO: 427 - RNA, 21 nt, artificial sequence
  source 1..21: mol_type = genomic RNA
aaccatgccacagagactcag

SEQ ID NO: 428 - RNA, 21 nt, artificial sequence
  source 1..21: mol_type = genomic RNA
tgttcccaaaccatgccacag

SEQ ID NO: 429 - RNA, 21 nt, artificial sequence
  source 1..21: mol_type = genomic RNA
tgtgttcccaaaccatgccac

SEQ ID NO: 430 - RNA, 21 nt, artificial sequence
  source 1..21: mol_type = genomic RNA
tgcttgtggtaatcggtaccc

SEQ ID NO: 431 - RNA, 21 nt, artificial sequence
  source 1..21: mol_type = genomic RNA
atggttgcttgtggtaatcgg

SEQ ID NO: 432 - RNA, 21 nt, artificial sequence
  source 1..21: mol_type = genomic RNA
actgagatcttggcctgccat

SEQ ID NO: 433 - RNA, 21 nt, artificial sequence
  source 1..21: mol_type = genomic RNA
tgactgagatcttggcctgcc

SEQ ID NO: 434 - RNA, 21 nt, artificial sequence
  source 1..21: mol_type = genomic RNA
tgaagggcgaatgactgagat

SEQ ID NO: 435 - RNA, 21 nt, artificial sequence
  source 1..21: mol_type = genomic RNA
agtactcagacaccacagccc

SEQ ID NO: 436 - RNA, 21 nt, artificial sequence
  source 1..21: mol_type = genomic RNA
acaatgtgctgctgtcagcac

SEQ ID NO: 437 - RNA, 21 nt, artificial sequence
  source 1..21: mol_type = genomic RNA
tccacagtgaaacaatgtgct

SEQ ID NO: 438 - RNA, 21 nt, artificial sequence
  source 1..21: mol_type = genomic RNA
ttgtcatccacagtgaaacaa

SEQ ID NO: 439 - RNA, 21 nt, artificial sequence
  source 1..21: mol_type = genomic RNA
ttccttgtcatccacagtgaa

SEQ ID NO: 440 - RNA, 21 nt, artificial sequence
  source 1..21: mol_type = genomic RNA
tgttccttgtcatccacagtg

SEQ ID NO: 441 - RNA, 21 nt, artificial sequence
  source 1..21: mol_type = genomic RNA
agtgttccttgtcatccacag

SEQ ID NO: 442 - RNA, 21 nt, artificial sequence
  source 1..21: mol_type = genomic RNA
ttgattgagtgttccttgtca

SEQ ID NO: 443 - RNA, 21 nt, artificial sequence
  source 1..21: mol_type = genomic RNA
tgaccttgattgagtgttcct

SEQ ID NO: 444 - RNA, 21 nt, artificial sequence
  source 1..21: mol_type = genomic RNA
ttctatctccaggtcccgctt

SEQ ID NO: 445 - RNA, 21 nt, artificial sequence
  source 1..21: mol_type = genomic RNA
acttctatctccaggtcccgc

SEQ ID NO: 446 - RNA, 21 nt, artificial sequence
  source 1..21: mol_type = genomic RNA
taggactacttctatctccag

SEQ ID NO: 447 - RNA, 21 nt, artificial sequence
  source 1..21: mol_type = genomic RNA
tgtagttggggtgaaatagga

SEQ ID NO: 448 - RNA, 21 nt, artificial sequence
  source 1..21: mol_type = genomic RNA
attcaggaattcctgcttctt

SEQ ID NO: 449 - RNA, 21 nt, artificial sequence
  source 1..21: mol_type = genomic RNA
taaaattcaggaattcctgct

SEQ ID NO: 450 - RNA, 21 nt, artificial sequence
  source 1..21: mol_type = genomic RNA
tcataaaattcaggaattcct

SEQ ID NO: 451 - RNA, 21 nt, artificial sequence
  source 1..21: mol_type = genomic RNA
tcatagtcataaaattcagga

SEQ ID NO: 452 - RNA, 21 nt, artificial sequence
  source 1..21: mol_type = genomic RNA
tgagcttgatcagggcaacgt

SEQ ID NO: 453 - RNA, 21 nt, artificial sequence
  source 1..21: mol_type = genomic RNA
tcttgagcttgatcagggcaa

SEQ ID NO: 454 - RNA, 21 nt, artificial sequence
  source 1..21: mol_type = genomic RNA
ttcttgagcttgatcagggca

SEQ ID NO: 455 - RNA, 21 nt, artificial sequence
  source 1..21: mol_type = genomic RNA
attcttgagcttgatcagggc

SEQ ID NO: 456 - RNA, 21 nt, artificial sequence
  source 1..21: mol_type = genomic RNA
ttattcttgagcttgatcagg

SEQ ID NO: 457 - RNA, 21 nt, artificial sequence
  source 1..21: mol_type = genomic RNA
tttcagcttattcttgagctt

SEQ ID NO: 458 - RNA, 21 nt, artificial sequence
  source 1..21: mol_type = genomic RNA
atgggcctgatagtctggcca

SEQ ID NO: 459 - RNA, 21 nt, artificial sequence
  source 1..21: mol_type = genomic RNA
aatgggcctgatagtctggcc

SEQ ID NO: 460 - RNA, 21 nt, artificial sequence
  source 1..21: mol_type = genomic RNA
aaatgggcctgatagtctggc

SEQ ID NO: 461 - RNA, 21 nt, artificial sequence
  source 1..21: mol_type = genomic RNA
acaaatgggcctgatagtctg

SEQ ID NO: 462 - RNA, 21 nt, artificial sequence
  source 1..21: mol_type = genomic RNA
tcgagttgttccctcggtgca

SEQ ID NO: 463 - RNA, 21 nt, artificial sequence
  source 1..21: mol_type = genomic RNA
agctcgagttgttccctcggt

SEQ ID NO: 464 - RNA, 21 nt, artificial sequence
  source 1..21: mol_type = genomic RNA
aagctcgagttgttccctcgg

SEQ ID NO: 465 - RNA, 21 nt, artificial sequence
  source 1..21: mol_type = genomic RNA
ttggaggaagcctcaaagctc

SEQ ID NO: 466 - RNA, 21 nt, artificial sequence
  source 1..21: mol_type = genomic RNA
agtggtagttggaggaagcct

SEQ ID NO: 467 - RNA, 21 nt, artificial sequence
  source 1..21: mol_type = genomic RNA
aagtggtagttggaggaagcc

SEQ ID NO: 468 - RNA, 21 nt, artificial sequence
  source 1..21: mol_type = genomic RNA
atcctgtgcagggagcagctc

SEQ ID NO: 469 - RNA, 21 nt, artificial sequence
  source 1..21: mol_type = genomic RNA
tttgatatcctgtgcagggag

SEQ ID NO: 470 - RNA, 21 nt, artificial sequence
  source 1..21: mol_type = genomic RNA
agagctttgatatcctgtgca

SEQ ID NO: 471 - RNA, 21 nt, artificial sequence
  source 1..21: mol_type = genomic RNA
acagagctttgatatcctgtg

SEQ ID NO: 472 - RNA, 21 nt, artificial sequence
  source 1..21: mol_type = genomic RNA
aacagagctttgatatcctgt

SEQ ID NO: 473 - RNA, 21 nt, artificial sequence
  source 1..21: mol_type = genomic RNA
aaacagagctttgatatcctg

SEQ ID NO: 474 - RNA, 21 nt, artificial sequence
  source 1..21: mol_type = genomic RNA
caaacagagctttgatatcct

SEQ ID NO: 475 - RNA, 21 nt, artificial sequence
  source 1..21: mol_type = genomic RNA
tcctcagacacaaacagagct

SEQ ID NO: 476 - RNA, 21 nt, artificial sequence
  source 1..21: mol_type = genomic RNA
agacctccttccgagtcagct

SEQ ID NO: 477 - RNA, 21 nt, artificial sequence
  source 1..21: mol_type = genomic RNA
tagacctccttccgagtcagc

SEQ ID NO: 478 - RNA, 21 nt, artificial sequence
  source 1..21: mol_type = genomic RNA
gtagacctccttccgagtcag

SEQ ID NO: 479 - RNA, 21 nt, artificial sequence
  source 1..21: mol_type = genomic RNA
atgtagacctccttccgagtc

SEQ ID NO: 480 - RNA, 21 nt, artificial sequence
  source 1..21: mol_type = genomic RNA
ttgatgtagacctccttccga

SEQ ID NO: 481 - RNA, 21 nt, artificial sequence
  source 1..21: mol_type = genomic RNA
cttgatgtagacctccttccg

SEQ ID NO: 482 - RNA, 21 nt, artificial sequence
  source 1..21: mol_type = genomic RNA
attcttgatgtagacctcctt

SEQ ID NO: 483 - RNA, 21 nt, artificial sequence
  source 1..21: mol_type = genomic RNA
cattcttgatgtagacctcct

SEQ ID NO: 484 - RNA, 21 nt, artificial sequence
  source 1..21: mol_type = genomic RNA
tttcttatccccattcttgat

SEQ ID NO: 485 - RNA, 21 nt, artificial sequence
  source 1..21: mol_type = genomic RNA
tgagcatctctctcacagctg

SEQ ID NO: 486 - RNA, 21 nt, artificial sequence
  source 1..21: mol_type = genomic RNA
ttgagcatctctctcacagct

SEQ ID NO: 487 - RNA, 21 nt, artificial sequence
  source 1..21: mol_type = genomic RNA
tattgagcatctctctcacag

SEQ ID NO: 488 - RNA, 21 nt, artificial sequence
  source 1..21: mol_type = genomic RNA
ttgactttgtcatagcctggg

SEQ ID NO: 489 - RNA, 21 nt, artificial sequence
  source 1..21: mol_type = genomic RNA
tccttgactttgtcatagcct

SEQ ID NO: 490 - RNA, 21 nt, artificial sequence
  source 1..21: mol_type = genomic RNA
agatgtccttgactttgtcat

SEQ ID NO: 491 - RNA, 21 nt, artificial sequence
  source 1..21: mol_type = genomic RNA
tcctccagtacaaaggaaccg

SEQ ID NO: 492 - RNA, 21 nt, artificial sequence
  source 1..21: mol_type = genomic RNA
tagggactcactcctccagta

SEQ ID NO: 493 - RNA, 21 nt, artificial sequence
  source 1..21: mol_type = genomic RNA
tctcttgtgaactatcaaggg

SEQ ID NO: 494 - RNA, 21 nt, artificial sequence
  source 1..21: mol_type = genomic RNA
aacgacttctcttgtgaacta

SEQ ID NO: 495 - RNA, 21 nt, artificial sequence
  source 1..21: mol_type = genomic RNA
tgaaacgacttctcttgtgaa

SEQ ID NO: 496 - RNA, 21 nt, artificial sequence
  source 1..21: mol_type = genomic RNA
aatgaaacgacttctcttgtg

SEQ ID NO: 497 - RNA, 21 nt, artificial sequence
  source 1..21: mol_type = genomic RNA
tgaatgaaacgacttctcttg

SEQ ID NO: 498 - RNA, 21 nt, artificial sequence
  source 1..21: mol_type = genomic RNA
ttgaatgaaacgacttctctt

SEQ ID NO: 499 - RNA, 21 nt, artificial sequence
  source 1..21: mol_type = genomic RNA
acttgaatgaaacgacttctc

SEQ ID NO: 500 - RNA, 21 nt, artificial sequence
  source 1..21: mol_type = genomic RNA
acaccaacttgaatgaaacga

SEQ ID NO: 501 - RNA, 21 nt, artificial sequence
  source 1..21: mol_type = genomic RNA
ttgatgtgaaagtctcgggcg

SEQ ID NO: 502 - RNA, 21 nt, artificial sequence
  source 1..21: mol_type = genomic RNA
aggttgatgtgaaagtctcgg

SEQ ID NO: 503 - RNA, 21 nt, artificial sequence
  source 1..21: mol_type = genomic RNA
agaggttgatgtgaaagtctc

SEQ ID NO: 504 - RNA, 21 nt, artificial sequence
  source 1..21: mol_type = genomic RNA
agtttctccttcagccagggc

SEQ ID NO: 505 - RNA, 21 nt, artificial sequence
  source 1..21: mol_type = genomic RNA
tggagtttctccttcagccag

SEQ ID NO: 506 - RNA, 21 nt, artificial sequence
  source 1..21: mol_type = genomic RNA
ttggagtttctccttcagcca

SEQ ID NO: 507 - RNA, 21 nt, artificial sequence
  source 1..21: mol_type = genomic RNA
atcttggagtttctccttcag

SEQ ID NO: 508 - RNA, 21 nt, artificial sequence
  source 1..21: mol_type = genomic RNA
atcctcatcttggagtttctc

SEQ ID NO: 509 - RNA, 21 nt, artificial sequence
  source 1..21: mol_type = genomic RNA
atagaaaacccaaatcctcat

SEQ ID NO: 510 - RNA, 21 nt, artificial sequence
  source 1..21: mol_type = genomic RNA
ttatagaaaacccaaatcctc

SEQ ID NO: 511 - DNA, 20 bp, artificial sequence
  source 1..20: mol_type = genomic DNA
gctgtgagagagatgctcaa

SEQ ID NO: 512 - DNA, 22 bp, artificial sequence
  source 1..22: mol_type = genomic DNA
gactcactcctccagtacaaag

SEQ ID NO: 513 - DNA, 27 bp, artificial sequence
  source 1..27: mol_type = genomic DNA
cccaggctatgacaaagtcaaggacat

SEQ ID NO: 514 - DNA, 19 bp, artificial sequence
  source 1..19: mol_type = genomic DNA
aagaaggtggtgaagcagg

SEQ ID NO: 515 - DNA, 18 bp, artificial sequence
  source 1..18: mol_type = genomic DNA
caaagtggtcgttgaggg

SEQ ID NO: 516 - DNA, 18 bp, artificial sequence
  source 1..18: mol_type = genomic DNA
caacagcgacacccactc

SEQ ID NO: 517 - DNA, 20 bp, artificial sequence
  source 1..20: mol_type = genomic DNA
cgttggctacccgtgatatt

SEQ ID NO: 518 - DNA, 22 bp, artificial sequence
  source 1..22: mol_type = genomic DNA
ctcgtcaagaaggcgatagaag

SEQ ID NO: 519 - DNA, 24 bp, artificial sequence
  source 1..24: mol_type = genomic DNA
ccgcttcctcgtgctttacggtat

SEQ ID NO: 520 - DNA, 20 bp, artificial sequence
  source 1..20: mol_type = genomic DNA
gccacgatatggtctcctga

SEQ ID NO: 521 - DNA, 20 bp, artificial sequence
  source 1..20: mol_type = genomic DNA
gagcttctctgtgacccagt

SEQ ID NO: 522 - DNA, 25 bp, artificial sequence
  source 1..25: mol_type = genomic DNA
cggcatcgctactcctctcatcaga

SEQ ID NO: 523 - DNA, 20 bp, artificial sequence
  source 1..20: mol_type = genomic DNA
tatgactccactcacggcaa

SEQ ID NO: 524 - DNA, 20 bp, artificial sequence
  source 1..20: mol_type = genomic DNA
tggaagatggtgatgggctt

SEQ ID NO: 525 - DNA, 21 bp, artificial sequence
  source 1..21: mol_type = genomic DNA
tctcggccttgactgtgccgt